European Patent Specification EP 3 737 403 B1, published January 3, 2024. Title: Modified Adenoviruses. Applicant: University College Cardiff Consultants Limited. The sequence listing filed with the application follows.

SEQUENCE LISTING (1 sequence)

SEQ ID NO: 1 - protein, 20 aa, Foot-and-mouth disease virus
NAVPNLRGDLQVLAQKVART